European Patent Application EP 4 570 819 A1, published June 18, 2025. Title: LONG-ACTING DUAL-AGONIST COMPOUND. Applicant: Chengdu Auda Biotechnology Co. , Ltd. Application US 19102413, filed August 7, 2023. The sequence listing filed with the application follows.

SEQUENCE LISTING (6 sequences)

SEQ ID NO: 1 - protein, 39 aa, synthetic construct
  MOD_RES 20: note = Lysine is modified with AEEA-AEEA-gamma Glu-eicosanedioic acid
  MOD_RES 2: note = X at location 2 is Aib
HXQGTFTSDYSKYLDEKKAKEFVEWLLEGGPSSGAPPPS

SEQ ID NO: 2 - protein, 39 aa, synthetic construct; identical to SEQ ID NO: 1
  MOD_RES 20: note = Lysine is modified with PEG5CH2CO-gamma Glu-eicosanedioic acid
  MOD_RES 2: note = X at location 2 is Aib

SEQ ID NO: 3 - protein, 39 aa, synthetic construct; identical to SEQ ID NO: 1
  MOD_RES 20: note = Lysine is modified with Gly-Gly-Ser-Gly-Ser-Gly-gamma Glu-eicosanedioic acid-gamma Glu-eicosanedioic acid
  MOD_RES 2: note = X at location 2 is Aib

SEQ ID NO: 4 - protein, 39 aa, synthetic construct; identical to SEQ ID NO: 1
  MOD_RES 20: note = Lysine is modified with Gly-Gly-Glu-Gly-Glu-Gly-gamma Glu-eicosanedioic acid
  MOD_RES 2: note = X at location 2 is Aib

SEQ ID NO: 5 - protein, 34 aa, synthetic construct
  MOD_RES 20: note = Lysine is modified with AEEA-AEEA-gamma Glu-eicosanedioic acid
  MOD_RES 2: note = X at location 2 is Aib
HXQGTFTSDYSKYLDEKKAKEFVEWLLEGGPSSG

SEQ ID NO: 6 - protein, 39 aa, synthetic construct
  VAR_SEQ 2: note = Amino acid at location 2 is selected from the group consisting of Aib, Acpr, Acp, Acpe and Ach.
  MOD_RES 20: note = Lysine is modified with R, and R is HO2C(CH2)n1CO-(AA4)n2-(PEGn3(CH2)n4CO)n5- or HO2C(CH2)n1CO-(AA4)n2-(AA5)n6-, wherein AA4 is selected from the group consisting of gamma-Glu, epsilon-Lys, beta-Ala, gamma-aminobutyric acid and 5-Ava, AA5 is selected from the group consisting of Gly, Ser, Thr, Asp, Glu, Aad, Lys, Orn, Dab and Dap. n1 is an integer selected from 10 to 20, n2 is an integer selected from 1 to 5, n3 is an integer selected from 1 to 30, n4 is an integer selected from 1 to 5, n5 is an integer selected from 1 to 10 and n6 is an integer selected from 1 to 10.
  VAR_SEQ 28: note = Amino acid at location 28 is Glu or Ser.
  MOD_RES 39: note = Amino acid at location 39 is linked with NH2 or OH
HXQGTFTSDYSKYLDEKKAKEFVEWLLXGGPSSGAPPPS